European Patent Specification EP 2 813 568 B1, published April 23, 2025. Title: Altered Fc region of antibody. Applicant: CHUGAI SEIYAKU KABUSHIKI KAISHA. The sequence listing filed with the application follows.

SEQUENCE LISTING (92 sequences)

SEQ ID NO: 1 - DNA, 2268 bp, Homo sapiens
aatatcttgcatgttacagatttcactgctcccaccagcttggagacaacatgtggttcttgacaactctgctcctttgggttccagttgatgggcaagtggacaccacaaaggcagtgatcactttgcagcctccatgggtcagcgtgttccaagaggaaaccgtaaccttgcactgtgaggtgctccatctgcctgggagcagctctacacagtggtttctcaatggcacagccactcagacctcgacccccagctacagaatcacctctgccagtgtcaatgacagtggtgaatacaggtgccagagaggtctctcagggcgaagtgaccccatacagctggaaatccacagaggctggctactactgcaggtctccagcagagtcttcacggaaggagaacctctggccttgaggtgtcatgcgtggaaggataagctggtgtacaatgtgctttactatcgaaatggcaaagcctttaagtttttccactggaattctaacctcaccattctgaaaaccaacataagtcacaatggcacctaccattgctcaggcatgggaaagcatcgctacacatcagcaggaatatctgtcactgtgaaagagctatttccagctccagtgctgaatgcatctgtgacatccccactcctggaggggaatctggtcaccctgagctgtgaaacaaagttgctcttgcagaggcctggtttgcagctttacttctccttctacatgggcagcaagaccctgcgaggcaggaacacatcctctgaataccaaatactaactgctagaagagaagactctgggttatactggtgcgaggctgccacagaggatggaaatgtccttaagcgcagccctgagttggagcttcaagtgcttggcctccagttaccaactcctgtctggtttcatgtccttttctatctggcagtgggaataatgtttttagtgaacactgttctctgggtgacaatacgtaaagaactgaaaagaaagaaaaagtgggatttagaaatctctttggattctggtcatgagaagaaggtaatttccagccttcaagaagacagacatttagaagaagagctgaaatgtcaggaacaaaaagaagaacagctgcaggaaggggtgcaccggaaggagccccagggggccacgtagcagcggctcagtgggtggccatcgatctggaccgtcccctgcccacttgctccccgtgagcactgcgtacaaacatccaaaagttcaacaacaccagaactgtgtgtctcatggtatgtaactcttaaagcaaataaatgaactgacttcaactgggatacatttggaaatgtggtcatcaaagatgacttgaaatgaggcctactctaaagaattcttgaaaaacttacaagtcaagcctagcctgataatcctattacatagtttgaaaaatagtattttatttctcagaacaaggtaaaaaggtgagtgggtgcatatgtacagaagattaagacagagaaacagacagaaagagacacacacacagccaggagtgggtagatttcagggagacaagagggaatagtatagacaataaggaaggaaatagtacttacaaatgactcctaagggactgtgagactgagagggctcacgcctctgtgttcaggatacttagttcatggcttttctctttgactttactaaaagagaatgtctccatacgcgttctaggcatacaagggggtaactcatgatgagaaatggatgtgttattcttgccctctcttttgaggctctctcataacccctctatttctagagacaacaaaaatgctgccagtcctaggcccctgccctgtaggaaggcagaatgtaactgttctgtttgtttaacgattaagtccaaatctccaagtgcggcactgcaaagagacgcttcaagtggggagaagcggcgataccatagagtccagatcttgcctccagagatttgctttaccttcctgattttctggttactaattagcttcaggatacgctgctctcatacttgggctgtagtttggagacaaaatattttcctgccactgtgtaacatagctgaggtaaaaactgaactatgtaaatgactctactaaaagtttagggaaaaaaaacaggaggagtatgacacaaaaaaaaaaaaaaaaaaaaaaaaaaaaaaaaaaaaaaaaaaaaaaaaaaaaaaaaaaaaaaaaaaaaaaaaaaaaaaaaaaaaaaaaaaaaa

SEQ ID NO: 2 - protein, 374 aa, Homo sapiens
MWFLTTLLLWVPVDGQVDTTKAVITLQPPWVSVFQEETVTLHCEVLHLPGSSSTQWFLNGTATQTSTPSYRITSASVNDSGEYRCQRGLSGRSDPIQLEIHRGWLLLQVSSRVFTEGEPLALRCHAWKDKLVYNVLYYRNGKAFKFFHWNSNLTILKTNISHNGTYHCSGMGKHRYTSAGISVTVKELFPAPVLNASVTSPLLEGNLVTLSCETKLLLQRPGLQLYFSFYMGSKTLRGRNTSSEYQILTARREDSGLYWCEAATEDGNVLKRSPELELQVLGLQLPTPVWFHVLFYLAVGIMFLVNTVLWVTIRKELKRKKKWDLEISLDSGHEKKVISSLQEDRHLEEELKCQEQKEEQLQEGVHRKEPQGAT

SEQ ID NO: 3 - DNA, 1396 bp, Homo sapiens
gggatgactatggagacccaaatgtctcagaatgtatgtcccagaaacctgtggctgcttcaaccattgacagttttgctgctgctggcttctgcagacagtcaagctgctcccccaaaggctgtgctgaaacttgagcccccgtggatcaacgtgctccaggaggactctgtgactctgacatgccagggggctcgcagccctgagagcgactccattcagtggttccacaatgggaatctcattcccacccacacgcagcccagctacaggttcaaggccaacaacaatgacagcggggagtacacgtgccagactggccagaccagcctcagcgaccctgtgcatctgactgtgctttccgaatggctggtgctccagacccctcacctggagttccaggagggagaaaccatcatgctgaggtgccacagctggaaggacaagcctctggtcaaggtcacattcttccagaatggaaaatcccagaaattctcccatttggatcccaccttctccatcccacaagcaaaccacagtcacagtggtgattaccactgcacaggaaacataggctacacgctgttctcatccaagcctgtgaccatcactgtccaagtgcccagcatgggcagctcttcaccaatgggggtcattgtggctgtggtcattgcgactgctgtagcagccattgttgctgctgtagtggccttgatctactgcaggaaaaagcggatttcagccaattccactgatcctgtgaaggctgcccaatttgagccacctggacgtcaaatgattgccatcagaaagagacaacttgaagaaaccaacaatgactatgaaacagctgacggcggctacatgactctgaaccccagggcacctactgacgatgataaaaacatctacctgactcttcctcccaacgaccatgtcaacagtaataactaaagagtaacgttatgccatgtggtcatactctcagcttgctgagtggatgacaaaaagaggggaattgttaaaggaaaatttaaatggagactggaaaaatcctgagcaaacaaaaccacctggcccttagaaatagctttaactttgcttaaactacaaacacaagcaaaacttcacggggtcatactacatacaagcataagcaaaacttaacttggatcatttctggtaaatgcttatgttagaaataagacaaccccagccaatcacaagcagcctactaacatataattaggtgactagggactttctaagaagatacctacccccaaaaaacaattatgtaattgaaaaccaaccgattgcctttattttgcttccacattttcccaataaatacttgcctgtgactaaaaaaaaaaaaaaaaaaaaaaaaaaaaaa

SEQ ID NO: 4 - protein, 316 aa, Homo sapiens
MTMETQMSQNVCPRNLWLLQPLTVLLLLASADSQAAPPKAVLKLEPPWINVLQEDSVTLTCQGARSPESDSIQWFHNGNLIPTHTQPSYRFKANNNDSGEYTCQTGQTSLSDPVHLTVLSEWLVLQTPHLEFQEGETIMLRCHSWKDKPLVKVTFFQNGKSQKFSHLDPTFSIPQANHSHSGDYHCTGNIGYTLFSSKPVTITVQVPSMGSSSPMGVIVAVVIATAVAAIVAAVVALIYCRKKRISANSTDPVKAAQFEPPGRQMIAIRKRQLEETNNDYETADGGYMTLNPRAPTDDDKNIYLTLPPNDHVNSNN

SEQ ID NO: 5 - DNA, 1497 bp, Homo sapiens
tgtgactgctgtgctctgggcgccagctcgctccagggagtgatgggaatcctgtcattcttacctgtccttgccactgagagtgactgggctgactgcaagtccccccagccttggggtcatatgcttctgtggacagctgtgctattcctggctcctgttgctgggacacctgcagctcccccaaaggctgtgctgaaactcgagccccagtggatcaacgtgctccaggaggactctgtgactctgacatgccgggggactcacagccctgagagcgactccattcagtggttccacaatgggaatctcattcccacccacacgcagcccagctacaggttcaaggccaacaacaatgacagcggggagtacacgtgccagactggccagaccagcctcagcgaccctgtgcatctgactgtgctttctgagtggctggtgctccagacccctcacctggagttccaggagggagaaaccatcgtgctgaggtgccacagctggaaggacaagcctctggtcaaggtcacattcttccagaatggaaaatccaagaaattttcccgttcggatcccaacttctccatcccacaagcaaaccacagtcacagtggtgattaccactgcacaggaaacataggctacacgctgtactcatccaagcctgtgaccatcactgtccaagctcccagctcttcaccgatggggatcattgtggctgtggtcactgggattgctgtagcggccattgttgctgctgtagtggccttgatctactgcaggaaaaagcggatttcagccaatcccactaatcctgatgaggctgacaaagttggggctgagaacacaatcacctattcacttctcatgcacccggatgctctggaagagcctgatgaccagaaccgtatttagtctccattgtcttgcattgggatttgagaagaaaatcagagagggaagatctggtatttcctggcctaaattccccttggggaggacagggagatgctgcagttccaaaagagaaggtttcttccagagtcatctacctgagtcctgaagctccctgtcctgaaagccacagacaatatggtcccaaataaccgactgcaccttctgtgcttcagctcttcttgacatcaaggctcttccgttccacatccacacagccaatccaattaatcaaaccactgttattaacagataatagcaacttgggaaatgcttatgttacaggttacgtgagaacaatcatgtaaatctatatgatttcagaaatgttaaaatagactaacctctaccagcacattaaaagtgattgtttctgggtgataaaattattgatgatttttattttctttatttttctataaagatcatatattacttttataataaaacattataaaaacaaaaaaaaaaaaaaaaaaaaaaaaaaaaaaaaaaaaaaaaaaaaaaaaaaaaaaaaaaaaaaaaaaaaaaaaaaaaaaa

SEQ ID NO: 6 - protein, 291 aa, Homo sapiens
MGILSFLPVLATESDWADCKSPQPWGHMLLWTAVLFLAPVAGTPAAPPKAVLKLEPQWINVLQEDSVTLTCRGTHSPESDSIQWFHNGNLIPTHTQPSYRFKANNNDSGEYTCQTGQTSLSDPVHLTVLSEWLVLQTPHLEFQEGETIVLRCHSWKDKPLVKVTFFQNGKSKKFSRSDPNFSIPQANHSHSGDYHCTGNIGYTLYSSKPVTITVQAPSSSPMGIIVAVVTGIAVAAIVAAVVALIYCRKKRISANPTNPDEADKVGAENTITYSLLMHPDALEEPDDQNRI

SEQ ID NO: 7 - DNA, 2137 bp, Homo sapiens
cttgtccactccagtgtggcatcatgtggcagctgctcctcccaactgctctgctacttctagtttcagctggcatgcggactgaagatctcccaaaggctgtggtgttcctggagcctcaatggtacagggtgctcgagaaggacagtgtgactctgaagtgccagggagcctactcccctgaggacaattccacacagtggtttcacaatgagagcctcatctcaagccaggcctcgagctacttcattgacgctgccacagttgacgacagtggagagtacaggtgccagacaaacctctccaccctcagtgacccggtgcagctagaagtccatatcggctggctgttgctccaggcccctcggtgggtgttcaaggaggaagaccctattcacctgaggtgtcacagctggaagaacactgctctgcataaggtcacatatttacagaatggcaaaggcaggaagtattttcatcataattctgacttctacattccaaaagccacactcaaagacagcggctcctacttctgcagggggcttgttgggagtaaaaatgtgtcttcagagactgtgaacatcaccatcactcaaggtttgtcagtgtcaaccatctcatcattctttccacctgggtaccaagtctctttctgcttggtgatggtactcctttttgcagtggacacaggactatatttctctgtgaagacaaacattcgaagctcaacaagagactggaaggaccataaatttaaatggagaaaggaccctcaagacaaatgacccccatcccatgggggtaataagagcagtagcagcagcatctctgaacatttctctggatttgcaaccccatcatcctcaggcctctctacaagcagcaggaaacatagaactcagagccagatcccttatccaactctcgacttttccttggtctccagtggaagggaaaagcccatgatcttcaagcagggaagccccagtgagtagctgcattcctagaaattgaagtttcagagctacacaaacactttttctgtcccaaccgttccctcacagcaaagcaacaatacaggctagggatggtaatcctttaaacatacaaaaattgctcgtgttataaattacccagtttagaggggaaaaaaaaacaattattcctaaataaatggataagtagaattaatggttgaggcaggaccatacagagtgtgggaactgctggggatctagggaattcagtgggaccaatgaaagcatggctgagaaatagcaggtagtccaggatagtctaagggaggtgttcccatctgagcccagagataagggtgtcttcctagaacattagccgtagtggaattaacaggaaatcatgagggtgacgtagaattgagtcttccaggggactctatcagaactggaccatctccaagtatataacgatgagtcctcttaatgctaggagtagaaaatggtcctaggaaggggactgaggattgcggtggggggtggggtggaaaagaaagtacagaacaaaccctgtgtcactgtcccaagttgctaagtgaacagaactatctcagcatcagaatgagaaagcctgagaagaaagaaccaaccacaagcacacaggaaggaaagcgcaggaggtgaaaatgctttcttggccagggtagtaagaattagaggttaatgcagggactgtaaaaccaccttttctgcttcaatatctaattcctgtgtagctttgttcattgcatttattaaacaaatgttgtataaccaatactaaatgtactactgagcttcgctgagttaagttatgaaactttcaaatccttcatcatgtcagttccaatgaggtggggatggagaagacaattgttgcttatgaaagaaagctttagctgtctctgttttgtaagctttaagcgcaacatttcttggttccaataaagcattttacaagatcttgcatgctactcttagatagaagatgggaaaaccatggtaataaaatatgaatgataaaaaaaaaaaaaaaaaaaaaaaaaaaaaaaaaaaaaaaaaaaaaaaaaaaaaaaaaaaaaaaaaaaaaaaaaaaaaaaaaaaaaaaaaaaaaaaaaaaa

SEQ ID NO: 8 - protein, 254 aa, Homo sapiens [sequence omitted]

SEQ ID NO: 9 - DNA, 820 bp, Homo sapiens
cactccagtgtggcatcatgtggcagctgctcctcccaactgctctgctacttctagtttcagctggcatgcggactgaagatctcccaaaggctgtggtgttcctggagcctcaatggtacagcgtgcttgagaaggacagtgtgactctgaagtgccagggagcctactcccctgaggacaattccacacagtggtttcacaatgagagcctcatctcaagccaggcctcgagctacttcattgacgctgccacagtcaacgacagtggagagtacaggtgccagacaaacctctccaccctcagtgacccggtgcagctagaagtccatatcggctggctgttgctccaggcccctcggtgggtgttcaaggaggaagaccctattcacctgaggtgtcacagctggaagaacactgctctgcataaggtcacatatttacagaatggcaaagacaggaagtattttcatcataattctgacttccacattccaaaagccacactcaaagatagcggctcctacttctgcagggggcttgttgggagtaaaaatgtgtcttcagagactgtgaacatcaccatcactcaaggtttggcagtgtcaaccatctcatcattctctccacctgggtaccaagtctctttctgcttggtgatggtactcctttttgcagtggacacaggactatatttctctgtgaagacaaacatttgaagctcaacaagagactggaaggaccataaacttaaatggagaaaggaccctcaagacaaatgacccccatcccatgggagtaataagagcagtggcagcag

SEQ ID NO: 10 - protein, 233 aa, Homo sapiens
MWQLLLPTALLLLVSAGMRTEDLPKAVVFLEPQWYSVLEKDSVTLKCQGAYSPEDNSTQWFHNESLISSQASSYFIDAATVNDSGEYRCQTNLSTLSDPVQLEVHIGWLLLQAPRWVFKEEDPIHLRCHSWKNTALHKVTYLQNGKDRKYFHHNSDFHIPKATLKDSGSYFCRGLVGSKNVSSETVNITITQGLAVSTISSFSPPGYQVSFCLVMVLLFAVDTGLYFSVKTNI

SEQ ID NO: 11 - protein, 330 aa, Artificial Sequence [sequence omitted]

SEQ ID NO: 12 - protein, 326 aa, Artificial Sequence
  an artificially synthesized sequence
ASTKGPSVFPLAPCSRSTSESTAALGCLVKDYFPEPVTVSWNSGALTSGVHTFPAVLQSSGLYSLSSVVTVPSSNFGTQTYTCNVDHKPSNTKVDKTVERKCCVECPPCPAPPVAGPSVFLFPPKPKDTLMISRTPEVTCVVVDVSHEDPEVQFNWYVDGVEVHNAKTKPREEQFNSTFRVVSVLTVVHQDWLNGKEYKCKVSNKGLPAPIEKTISKTKGQPREPQVYTLPPSREEMTKNQVSLTCLVKGFYPSDIAVEWESNGQPENNYKTTPPMLDSDGSFFLYSKLTVDKSRWQQGNVFSCSVMHEALHNHYTQKSLSLSPGK

SEQ ID NO: 13 - protein, 377 aa, Artificial Sequence
  an artificially synthesized sequence
ASTKGPSVFPLAPCSRSTSGGTAALGCLVKDYFPEPVTVSWNSGALTSGVHTFPAVLQSSGLYSLSSVVTVPSSSLGTQTYTCNVNHKPSNTKVDKRVELKTPLGDTTHTCPRCPEPKSCDTPPPCPRCPEPKSCDTPPPCPRCPEPKSCDTPPPCPRCPAPELLGGPSVFLFPPKPKDTLMISRTPEVTCVVVDVSHEDPEVQFKWYVDGVEVHNAKTKPREEQYNSTFRVVSVLTVLHQDWLNGKEYKCKVSNKALPAPIEKTISKTKGQPREPQVYTLPPSREEMTKNQVSLTCLVKGFYPSDIAVEWESSGQPENNYNTTPPMLDSDGSFFLYSKLTVDKSRWQQGNIFSCSVMHEALHNRFTQKSLSLSPGK

SEQ ID NO: 14 - protein, 327 aa, Artificial Sequence
  an artificially synthesized sequence
ASTKGPSVFPLAPCSRSTSESTAALGCLVKDYFPEPVTVSWNSGALTSGVHTFPAVLQSSGLYSLSSVVTVPSSSLGTKTYTCNVDHKPSNTKVDKRVESKYGPPCPSCPAPEFLGGPSVFLFPPKPKDTLMISRTPEVTCVVVDVSQEDPEVQFNWYVDGVEVHNAKTKPREEQFNSTYRVVSVLTVLHQDWLNGKEYKCKVSNKGLPSSIEKTISKAKGQPREPQVYTLPPSQEEMTKNQVSLTCLVKGFYPSDIAVEWESNGQPENNYKTTPPVLDSDGSFFLYSRLTVDKSRWQEGNVFSCSVMHEALHNHYTQKSLSLSLGK

SEQ ID NO: 15 - protein, 328 aa, Artificial Sequence
  an artificially synthesized sequence
ASTKGPSVFPLAPSSKSTSGGTAALGCLVKDYFPEPVTVSWNSGALTSGVHTFPAVLQSSGLYSLSSVVTVPSSSLGTQTYICNVNHKPSNTKVDKKVEPKSCDKTHTCPPCPAPELLGGPSVFLFPPKPKDTLMISRTPEVTCVVVDVSHEDPEVKFNWYVDGVEVHNAKTKPREEQYNSTYRVVSVLTVLHQDWLNGKEYKCKVSNKALPAPIEKTISKAKGQPREPQVYTLPPSRDELTKNQVSLTCLVKGFYPSDIAVEWESNGQPENNYKTTPPVLDSDGSFFLYSKLTVDKSRWQQGNVFSCSVMHEALHNHYTQKSLSLSP

SEQ ID NO: 16 - protein, 328 aa, Artificial Sequence
  an artificially synthesized sequence
ASTKGPSVFPLAPSSKSTSGGTAALGCLVKDYFPEPVTVSWNSGALTSGVHTFPAVLQSSGLYSLSSVVTVPSSSLGTQTYICNVNHKPSNTKVDKKVEPKSCDKTHTCPPCPAPELLGGPSVFLFPPKPKDTLMISRTPEVTCVVVDVSHEDPEVKFNWYVDGVEVHNAKTKPREEQYNSTYRVVSVLTVLHQDWLNGKEYKCKVSNKALPAPIEKTISKAKGQPREPQVYTLPPSRDELTKNQVSLTCLVKGFYPSDIAVEWESNGQPENNYKTTPPVLDSDGSFFLYSKLTVDKSRWQQGNVFSCSVMHEALHNHYTQESLSLSP

SEQ ID NO: 17 - protein, 115 aa, Artificial Sequence
  an artificially synthesized sequence
QVQLVQSGAEVKKPGASVTVSCKASGYTFTDYEMHWIRQPPGEGLEWIGAIDPKTGDTAYSESFQDRVTLTADKSTSTAYMELSSLTSEDTAVYYCTRFYSYTYWGQGTLVTVSS

SEQ ID NO: 18 - protein, 112 aa, Artificial Sequence
  an artificially synthesized sequence
DIVMTQSPLSLPVTPGEPASISCQASESLVHSNRNTYLHWYLQKPGQSPQLLIYKVSNRFSGVPDRFSGSGSGTDFTLKISRVEAEDVGVYYCSQNTHVPPTFGQGTKVEIE

SEQ ID NO: 19 - protein, 107 aa, Artificial Sequence [sequence omitted]

SEQ ID NO: 20 - protein, 119 aa, Artificial Sequence [sequence omitted]

SEQ ID NO: 21 - protein, 107 aa, Artificial Sequence [sequence omitted]

SEQ ID NO: 22 - protein, 443 aa, Artificial Sequence
  an artificially synthesized sequence
QVQLVQSGAEVKKPGASVTVSCKASGYTFTDYEMHWIRQPPGEGLEWIGAIDPKTGDTAYSESFQDRVTLTADKSTSTAYMELSSLTSEDTAVYYCTRFYSYTYWGQGTLVTVSSASTKGPSVFPLAPSSKSTSGGTAALGCLVKDYFPEPVTVSWNSGALTSGVHTFPAVLQSSGLYSLSSVVTVPSSSLGTQTYICNVNHKPSNTKVDKKVEPKSCDKTHTCPPCPAPELLGGPSVFLFPPKPKDTLMISRTPEVTCVVVDVSHEDPEVKFNWYVDGVEVHNAKTKPREEQYNSTYRVVSVLTVLHQDWLNGKEYKCKVSNKALPAPIEKTISKAKGQPREPQVYTLPPSRDELTKNQVSLTCLVKGFYPSDIAVEWESNGQPENNYKTTPPVLDSDGSFFLYSKLTVDKSRWQQGNVFSCSVMHEALHNHYTQKSLSLSP

SEQ ID NO: 23 - protein, 447 aa, Artificial Sequence
  an artificially synthesized sequence
QVQLQESGPGLVRPSQTLSLTCTVSGYSITSDHAWSWVRQPPGRGLEWIGYISYSGITTYNPSLKSRVTMLRDTSKNQFSLRLSSVTAADTAVYYCARSLARTTAMDYWGQGSLVTVSSASTKGPSVFPLAPSSKSTSGGTAALGCLVKDYFPEPVTVSWNSGALTSGVHTFPAVLQSSGLYSLSSVVTVPSSSLGTQTYICNVNHKPSNTKVDKKVEPKSCDKTHTCPPCPAPELLGGPSVFLFPPKPKDTLMISRTPEVTCVVVDVSHEDPEVKFNWYVDGVEVHNAKTKPREEQYNSTYRVVSVLTVLHQDWLNGKEYKCKVSNKALPAPIEKTISKAKGQPREPQVYTLPPSRDELTKNQVSLTCLVKGFYPSDIAVEWESNGQPENNYKTTPPVLDSDGSFFLYSKLTVDKSRWQQGNVFSCSVMHEALHNHYTQKSLSLSP

SEQ ID NO: 24 - protein, 328 aa, Artificial Sequence
  an artificially synthesized sequence
ASTKGPSVFPLAPSSKSTSGGTAALGCLVKDYFPEPVTVSWNSGALTSGVHTFPAVLQSSGLYSLSSVVTVPSSSLGTQTYICNVNHKPSNTKVDKKVEPKSCDKTHTCPPCPAPELLGGPSVFCFPPKPKDTLMISRTPEVTCVVVDVSHEDPEVKFNWYVDGVEVHNAKTKPREEQYNSTYRVVSVLTVLHQDWLNGKEYKCKVSNKALPAPIECTISKAKGQPREPQVYTLPPSRDELTKNQVSLTCLVKGFYPSDIAVEWESNGQPENNYKTTPPVLDSDGSFFLYSKLTVDKSRWQQGNVFSCSVMHEALHNHYTQKSLSLSP

SEQ ID NO: 25 - protein, 328 aa, Artificial Sequence
  an artificially synthesized sequence
ASTKGPSVFPLAPSSKSTSGGTAALGCLVKDYFPEPVTVSWNSGALTSGVHTFPAVLQSSGLYSLSSVVTVPSSSLGTQTYICNVNHKPSNTKVDKKVEPKSCDKTHTCPPCPAPELLGGPSCFLFPPKPKDTLMISRTPEVTCVVVDVSHEDPEVKFNWYVDGVEVHNAKTKPREEQYNSTYRVVSVLTVLHQDWLNGKEYKCKVSNKALPAPIECTISKAKGQPREPQVYTLPPSRDELTKNQVSLTCLVKGFYPSDIAVEWESNGQPENNYKTTPPVLDSDGSFFLYSKLTVDKSRWQQGNVFSCSVMHEALHNHYTQKSLSLSP

SEQ ID NO: 26 - protein, 328 aa, Artificial Sequence
  an artificially synthesized sequence
ASTKGPSVFPLAPSSKSTSGGTAALGCLVKDYFPEPVTVSWNSGALTSGVHTFPAVLQSSGLYSLSSVVTVPSSSLGTQTYICNVNHKPSNTKVDKKVEPKSCDKTHTCPPCPAPEILGGPSVFLFPPKPKDTLMISRTPEVTCVVVDVSHEDPEVKFNWYVDGVEVHNAKTKPREEQYNSTYRVVSVLTVLHQDWLNGKEYKCKVSNKALPAPIEKTISKAKGQPREPQVYTLPPSRDELTKNQVSLTCLVKGFYPSDIAVEWESNGQPENNYKTTPPVLDSDGSFFLYSKLTVDKSRWQQGNVFSCSVMHEALHNHYTQKSLSLSP

SEQ ID NO: 27 - protein, 328 aa, Artificial Sequence
  an artificially synthesized sequence
ASTKGPSVFPLAPSSKSTSGGTAALGCLVKDYFPEPVTVSWNSGALTSGVHTFPAVLQSSGLYSLSSVVTVPSSSLGTQTYICNVNHKPSNTKVDKKVEPKSCDKTHTCPPCPAPELLGGPSVFLFPPKPKDTLMISRTPEVTCVVVDISQDEPEVKFNWYVDGVEVHNAKTKPREEQYNSTYRVVSVLTVLHQDWLNGKEYKCKVSNKALPAPIEKTISKAKGQPREPQVYTLPPSRDELTKNQVSLTCLVKGFYPSDIAVEWESNGQPENNYKTTPPVLDSDGSFFLYSKLTVDKSRWQQGNVFSCSVMHEALHNHYTQKSLSLSP

SEQ ID NO: 28 - protein, 328 aa, Artificial Sequence
  an artificially synthesized sequence
ASTKGPSVFPLAPSSKSTSGGTAALGCLVKDYFPEPVTVSWNSGALTSGVHTFPAVLQSSGLYSLSSVVTVPSSSLGTQTYICNVNHKPSNTKVDKKVEPKSCDKTHTCPPCPAPELLGGPSVFLFPPKPKDTLMISRTPEVTCVVVDVSHEDPEVKFNWYVDGVEVHNAKTKPREEMYNSTYRVVSVLTVLHQDWLNGKEYKCKVSNKALPAPIEKTISKAKGQPREPQVYTLPPSRDELTKNQVSLTCLVKGFYPSDIAVEWESNGQPENNYKTTPPVLDSDGSFFLYSKLTVDKSRWQQGNVFSCSVMHEALHNHYTQKSLSLSP

SEQ ID NO: 29 - protein, 328 aa, Artificial Sequence
  an artificially synthesized sequence
ASTKGPSVFPLAPSSKSTSGGTAALGCLVKDYFPEPVTVSWNSGALTSGVHTFPAVLQSSGLYSLSSVVTVPSSSLGTQTYICNVNHKPSNTKVDKKVEPKSCDKTHTCPPCPAPELLGGPSVFLFPPKPKDTLMISRTPEVTCVVVDVSHEDPEVKFNWYVDGVEVHNAKTKPREEMYNSTERVVSVLTVLHQDWLNGKEYKCKVSNKALPAPIEKTISKAKGQPREPQVYTLPPSRDELTKNQVSLTCLVKGFYPSDIAVEWESNGQPENNYKTTPPVLDSDGSFFLYSKLTVDKSRWQQGNVFSCSVMHEALHNHYTQKSLSLSP

SEQ ID NO: 30 - protein, 328 aa, Artificial Sequence
  an artificially synthesized sequence
ASTKGPSVFPLAPSSKSTSGGTAALGCLVKDYFPEPVTVSWNSGALTSGVHTFPAVLQSSGLYSLSSVVTVPSSSLGTQTYICNVNHKPSNTKVDKKVEPKSCDKTHTCPPCPAPELLGGPSVFLFPPKPKDTLMISRTPEVTCVVVDVSHEDPEVKFNWYVDGVEVHNAKTKPREELYNSTYRVVSVLTVLHQDWLNGKEYKCKVSNKALPAPIEKTISKAKGQPREPQVYTLPPSRDELTKNQVSLTCLVKGFYPSDIAVEWESNGQPENNYKTTPPVLDSDGSFFLYSKLTVDKSRWQQGNVFSCSVMHEALHNHYTQKSLSLSP

SEQ ID NO: 31 - protein, 328 aa, Artificial Sequence
  an artificially synthesized sequence
ASTKGPSVFPLAPSSKSTSGGTAALGCLVKDYFPEPVTVSWNSGALTSGVHTFPAVLQSSGLYSLSSVVTVPSSSLGTQTYICNVNHKPSNTKVDKKVEPKSCDKTHTCPPCPAPELLGGPSVFLFPPKPKDTLMISRTPEVTCVVVDVSHEDPEVKFNWYVDGVEVHNAKTKPREEQYNSTYRVVSVLTVLHQDWLNGKEYKCKVSNSALPHPIEKTISKAKGQPREPQVYTLPPSRDELTKNQVSLTCLVKGFYPSDIAVEWESNGQPENNYKTTPPVLDSDGSFFLYSKLTVDKSRWQQGNVFSCSVMHEALHNHYTQKSLSLSP

SEQ ID NO: 32 - protein, 328 aa, Artificial Sequence
  an artificially synthesized sequence
ASTKGPSVFPLAPSSKSTSGGTAALGCLVKDYFPEPVTVSWNSGALTSGVHTFPAVLQSSGLYSLSSVVTVPSSSLGTQTYICNVNHKPSNTKVDKKVEPKSCDKTHTCPPCPAPELLGGPSVFLFPPKPKDTLMISRTPEVTCVVVDVSHEDPEVKFNWYVDGVEVHNAKTKPREEQYNSTYRVVSVLTVLHQDWLNGKEYKCKVHNSALPHPIEKTISKAKGQPREPQVYTLPPSRDELTKNQVSLTCLVKGFYPSDIAVEWESNGQPENNYKTTPPVLDSDGSFFLYSKLTVDKSRWQQGNVFSCSVMHEALHNHYTQKSLSLSP

SEQ ID NO: 33 - protein, 328 aa, Artificial Sequence
  an artificially synthesized sequence
ASTKGPSVFPLAPSSKSTSGGTAALGCLVKDYFPEPVTVSWNSGALTSGVHTFPAVLQSSGLYSLSSVVTVPSSSLGTQTYICNVNHKPSNTKVDKKVEPKSCDKTHTCPPCPAPELLGGPSVFLFPPKPKDTLMISRTPEVTCVVVDVSHEDPEVKFNWYVDGVEVHNAKTKPREEQYNSTYRVVSVLTVLHQDWLNGKEYKCKVSNAALPYPIEKTISKAKGQPREPQVYTLPPSRDELTKNQVSLTCLVKGFYPSDIAVEWESNGQPENNYKTTPPVLDSDGSFFLYSKLTVDKSRWQQGNVFSCSVMHEALHNHYTQKSLSLSP

SEQ ID NO: 34 - protein, 328 aa, Artificial Sequence
  an artificially synthesized sequence
ASTKGPSVFPLAPSSKSTSGGTAALGCLVKDYFPEPVTVSWNSGALTSGVHTFPAVLQSSGLYSLSSVVTVPSSSLGTQTYICNVNHKPSNTKVDKKVEPKSCDKTHTCPPCPAPEKKGGPSVFLFPPKPKDTLMISRTPEVTCVVVDVSHEDPEVKFNWYVDGVEVHNAKTKPREEQYNSTYRVVSVLTVLHQDWLNGKEYKCKVSNKALPAPIEKTISKAKGQPREPQVYTLPPSRDELTKNQVSLTCLVKGFYPSDIAVEWESNGQPENNYKTTPPVLDSDGSFFLYSKLTVDKSRWQQGNVFSCSVMHEALHNHYTQKSLSLSP

SEQ ID NO: 35 - protein, 328 aa, Artificial Sequence
  an artificially synthesized sequence
ASTKGPSVFPLAPSSKSTSGGTAALGCLVKDYFPEPVTVSWNSGALTSGVHTFPAVLQSSGLYSLSSVVTVPSSSLGTQTYICNVNHKPSNTKVDKKVEPKSCDKTHTCPPCPAPEKRGGPSVFLFPPKPKDTLMISRTPEVTCVVVDVSHEDPEVKFNWYVDGVEVHNAKTKPREEQYNSTYRVVSVLTVLHQDWLNGKEYKCKVSNKALPAPIEKTISKAKGQPREPQVYTLPPSRDELTKNQVSLTCLVKGFYPSDIAVEWESNGQPENNYKTTPPVLDSDGSFFLYSKLTVDKSRWQQGNVFSCSVMHEALHNHYTQKSLSLSP

SEQ ID NO: 36 - protein, 328 aa, Artificial Sequence
  an artificially synthesized sequence
ASTKGPSVFPLAPSSKSTSGGTAALGCLVKDYFPEPVTVSWNSGALTSGVHTFPAVLQSSGLYSLSSVVTVPSSSLGTQTYICNVNHKPSNTKVDKKVEPKSCDKTHTCPPCPAPERKGGPSVFLFPPKPKDTLMISRTPEVTCVVVDVSHEDPEVKFNWYVDGVEVHNAKTKPREEQYNSTYRVVSVLTVLHQDWLNGKEYKCKVSNKALPAPIEKTISKAKGQPREPQVYTLPPSRDELTKNQVSLTCLVKGFYPSDIAVEWESNGQPENNYKTTPPVLDSDGSFFLYSKLTVDKSRWQQGNVFSCSVMHEALHNHYTQKSLSLSP

SEQ ID NO: 37 - protein, 328 aa, Artificial Sequence
  an artificially synthesized sequence
ASTKGPSVFPLAPSSKSTSGGTAALGCLVKDYFPEPVTVSWNSGALTSGVHTFPAVLQSSGLYSLSSVVTVPSSSLGTQTYICNVNHKPSNTKVDKKVEPKSCDKTHTCPPCPAPERRGGPSVFLFPPKPKDTLMISRTPEVTCVVVDVSHEDPEVKFNWYVDGVEVHNAKTKPREEQYNSTYRVVSVLTVLHQDWLNGKEYKCKVSNKALPAPIEKTISKAKGQPREPQVYTLPPSRDELTKNQVSLTCLVKGFYPSDIAVEWESNGQPENNYKTTPPVLDSDGSFFLYSKLTVDKSRWQQGNVFSCSVMHEALHNHYTQKSLSLSP

SEQ ID NO: 38 - protein, 328 aa, Artificial Sequence
  an artificially synthesized sequence
ASTKGPSVFPLAPSSKSTSGGTAALGCLVKDYFPEPVTVSWNSGALTSGVHTFPAVLQSSGLYSLSSVVTVPSSSLGTQTYICNVNHKPSNTKVDKKVEPKSCDKTHTCPPCPAPELLGGPSVFLFPPKPKDTLMISRTPEVTCVVVDVPMEFPEVKFNWYVDGVEVHNAKTKPREEQYNSTYRVVSVLTVLHQDWLNGKEYKCKVSNKALPAPIEKTISKAKGQPREPQVYTLPPSRDELTKNQVSLTCLVKGFYPSDIAVEWESNGQPENNYKTTPPVLDSDGSFFLYSKLTVDKSRWQQGNVFSCSVMHEALHNHYTQKSLSLSP

SEQ ID NO: 39 - protein, 328 aa, Artificial Sequence
  an artificially synthesized sequence
ASTKGPSVFPLAPSSKSTSGGTAALGCLVKDYFPEPVTVSWNSGALTSGVHTFPAVLQSSGLYSLSSVVTVPSSSLGTQTYICNVNHKPSNTKVDKKVEPKSCDKTHTCPPCPAPELLGGPSVFLFPPKPKDTLMISRTPEVTCVVVDVSMEFPEVKFNWYVDGVEVHNAKTKPREEQYNSTYRVVSVLTVLHQDWLNGKEYKCKVSNKALPAPIEKTISKAKGQPREPQVYTLPPSRDELTKNQVSLTCLVKGFYPSDIAVEWESNGQPENNYKTTPPVLDSDGSFFLYSKLTVDKSRWQQGNVFSCSVMHEALHNHYTQKSLSLSP

SEQ ID NO: 40 - protein, 328 aa, Artificial Sequence
  an artificially synthesized sequence
ASTKGPSVFPLAPSSKSTSGGTAALGCLVKDYFPEPVTVSWNSGALTSGVHTFPAVLQSSGLYSLSSVVTVPSSSLGTQTYICNVNHKPSNTKVDKKVEPKSCDKTHTCPPCPAPELLGGPSVFLFPPKPKDTLMISRTPEVTCVVVDVSKEFPEVKFNWYVDGVEVHNAKTKPREEQYNSTYRVVSVLTVLHQDWLNGKEYKCKVSNKALPAPIEKTISKAKGQPREPQVYTLPPSRDELTKNQVSLTCLVKGFYPSDIAVEWESNGQPENNYKTTPPVLDSDGSFFLYSKLTVDKSRWQQGNVFSCSVMHEALHNHYTQKSLSLSP

SEQ ID NO: 41 - protein, 328 aa, Artificial Sequence
  an artificially synthesized sequence
ASTKGPSVFPLAPSSKSTSGGTAALGCLVKDYFPEPVTVSWNSGALTSGVHTFPAVLQSSGLYSLSSVVTVPSSSLGTQTYICNVNHKPSNTKVDKKVEPKSCDKTHTCPPCPAPELLGGPSVFLFPPKPKDTLMISRTPEVTCVVVDVSHEDPEVKFNWYVDGVEVHNAKTKPREEMGNGTYRVVSVLTVLHQDWLNGKEYKCKVSNKALPAPIEKTISKAKGQPREPQVYTLPPSRDELTKNQVSLTCLVKGFYPSDIAVEWESNGQPENNYKTTPPVLDSDGSFFLYSKLTVDKSRWQQGNVFSCSVMHEALHNHYTQKSLSLSP

SEQ ID NO: 42 - protein, 328 aa, Artificial Sequence
  an artificially synthesized sequence
ASTKGPSVFPLAPSSKSTSGGTAALGCLVKDYFPEPVTVSWNSGALTSGVHTFPAVLQSSGLYSLSSVVTVPSSSLGTQTYICNVNHKPSNTKVDKKVEPKSCDKTHTCPPCPAPELLGGPKVFLFPPKPKDTLMISRTPEVTCVVVDVSHEDPEVKFNWYVDGVEVHNAKTKPREEQYNSTYRVVSVLTVLHQDWLNGKEYKCKVSGKALPAPIEKTISKAKGQPREPQVYTLPPSRDELTKNQVSLTCLVKGFYPSDIAVEWESNGQPENNYKTTPPVLDSDGSFFLYSKLTVDKSRWQQGNVFSCSVMHEALHNHYTQKSLSLSP

SEQ ID NO: 43 - protein, 328 aa, Artificial Sequence
  an artificially synthesized sequence
ASTKGPSVFPLAPSSKSTSGGTAALGCLVKDYFPEPVTVSWNSGALTSGVHTFPAVLQSSGLYSLSSVVTVPSSSLGTQTYICNVNHKPSNTKVDKKVEPKSCDKTHTCPPCPAPELLGGPKVFLFPPKPKDTLMISRTPEVTCVVVDVSHEDPEVKFNWYVDGVEVHNAKTKPREEQYNSTYRVVSVLTVLHQDWLNGKEYKCKVSMKALPAPIEKTISKAKGQPREPQVYTLPPSRDELTKNQVSLTCLVKGFYPSDIAVEWESNGQPENNYKTTPPVLDSDGSFFLYSKLTVDKSRWQQGNVFSCSVMHEALHNHYTQKSLSLSP

SEQ ID NO: 44 - protein, 328 aa, Artificial Sequence
  an artificially synthesized sequence
ASTKGPSVFPLAPSSKSTSGGTAALGCLVKDYFPEPVTVSWNSGALTSGVHTFPAVLQSSGLYSLSSVVTVPSSSLGTQTYICNVNHKPSNTKVDKKVEPKSCDKTHTCPPCPAPELLGGPKVFLFPPKPKDTLMISRTPEVTCVVVDVSHEDPEVKFNWYVDGVEVHNAKTKPREEQYNSTYRVVSVLTVLHQDWLNGKEYKCKVSHKALPAPIEKTISKAKGQPREPQVYTLPPSRDELTKNQVSLTCLVKGFYPSDIAVEWESNGQPENNYKTTPPVLDSDGSFFLYSKLTVDKSRWQQGNVFSCSVMHEALHNHYTQKSLSLSP

SEQ ID NO: 45 - protein, 328 aa, Artificial Sequence
  an artificially synthesized sequence
ASTKGPSVFPLAPSSKSTSGGTAALGCLVKDYFPEPVTVSWNSGALTSGVHTFPAVLQSSGLYSLSSVVTVPSSSLGTQTYICNVNHKPSNTKVDKKVEPKSCDKTHTCPPCPAPELLGGPSVFLFPPKPKDTLMISRTPEVTCVVVDVSHEDPEVKFNWYVDGVEVHNAKTKPREEMYNSTYRVVSVLTVLHQDWLNGKEYKCKVSNSALPHPIEKTISKAKGQPREPQVYTLPPSRDELTKNQVSLTCLVKGFYPSDIAVEWESNGQPENNYKTTPPVLDSDGSFFLYSKLTVDKSRWQQGNVFSCSVMHEALHNHYTQKSLSLSP

SEQ ID NO: 46 - protein, 328 aa, Artificial Sequence
  an artificially synthesized sequence
ASTKGPSVFPLAPSSKSTSGGTAALGCLVKDYFPEPVTVSWNSGALTSGVHTFPAVLQSSGLYSLSSVVTVPSSSLGTQTYICNVNHKPSNTKVDKKVEPKSCDKTHTCPPCPAPELLGGPSVFLFPPKPKDTLMISRTPEVTCVVVDVSHEDPEVKFNWYVDGVEVHNAKTKPREEMYNSTYRVVSVLTVLHQDWLNGKEYKCKVSNAALPYPIEKTISKAKGQPREPQVYTLPPSRDELTKNQVSLTCLVKGFYPSDIAVEWESNGQPENNYKTTPPVLDSDGSFFLYSKLTVDKSRWQQGNVFSCSVMHEALHNHYTQKSLSLSP

SEQ ID NO: 47 - protein, 328 aa, Artificial Sequence
  an artificially synthesized sequence
ASTKGPSVFPLAPSSKSTSGGTAALGCLVKDYFPEPVTVSWNSGALTSGVHTFPAVLQSSGLYSLSSVVTVPSSSLGTQTYICNVNHKPSNTKVDKKVEPKSCDKTHTCPPCPAPELLGGPSVFLFPPKPKDTLMISRTPEVTCVVVDVSHEDPEVKFNWYVDGVEVHNAKTKPREELYNSTYRVVSVLTVLHQDWLNGKEYKCKVSNSALPHPIEKTISKAKGQPREPQVYTLPPSRDELTKNQVSLTCLVKGFYPSDIAVEWESNGQPENNYKTTPPVLDSDGSFFLYSKLTVDKSRWQQGNVFSCSVMHEALHNHYTQKSLSLSP

SEQ ID NO: 48 - protein, 328 aa, Artificial Sequence
  an artificially synthesized sequence
ASTKGPSVFPLAPSSKSTSGGTAALGCLVKDYFPEPVTVSWNSGALTSGVHTFPAVLQSSGLYSLSSVVTVPSSSLGTQTYICNVNHKPSNTKVDKKVEPKSCDKTHTCPPCPAPELLGGPSVFLFPPKPKDTLMISRTPEVTCVVVDVSHEDPEVKFNWYVDGVEVHNAKTKPREELYNSTYRVVSVLTVLHQDWLNGKEYKCKVSNAALPYPIEKTISKAKGQPREPQVYTLPPSRDELTKNQVSLTCLVKGFYPSDIAVEWESNGQPENNYKTTPPVLDSDGSFFLYSKLTVDKSRWQQGNVFSCSVMHEALHNHYTQKSLSLSP

SEQ ID NO: 49 - protein, 328 aa, Artificial Sequence
  an artificially synthesized sequence
ASTKGPSVFPLAPSSKSTSGGTAALGCLVKDYFPEPVTVSWNSGALTSGVHTFPAVLQSSGLYSLSSVVTVPSSSLGTQTYICNVNHKPSNTKVDKKVEPKSCDKTHTCPPCPAPELLGGPSVFLFPPKPKDTLMISRTPEVTCVVVDVSHEDPEVKFNWYVDGVEVHNAKTKPREEMYNSTYRVVSVLTVLHQDWLNGKEYKCKVSNSALPYPIEKTISKAKGQPREPQVYTLPPSRDELTKNQVSLTCLVKGFYPSDIAVEWESNGQPENNYKTTPPVLDSDGSFFLYSKLTVDKSRWQQGNVFSCSVMHEALHNHYTQKSLSLSP

SEQ ID NO: 50 - protein, 328 aa, Artificial Sequence
  an artificially synthesized sequence
ASTKGPSVFPLAPSSKSTSGGTAALGCLVKDYFPEPVTVSWNSGALTSGVHTFPAVLQSSGLYSLSSVVTVPSSSLGTQTYICNVNHKPSNTKVDKKVEPKSCDKTHTCPPCPAPELLGGPSVFLFPPKPKDTLMISRTPEVTCVVVDVSHEDPEVKFNWYVDGVEVHNAKTKPREEMYNSTYRVVSVLTVLHQDWLNGKEYKCKVSNAALPHPIEKTISKAKGQPREPQVYTLPPSRDELTKNQVSLTCLVKGFYPSDIAVEWESNGQPENNYKTTPPVLDSDGSFFLYSKLTVDKSRWQQGNVFSCSVMHEALHNHYTQKSLSLSP

SEQ ID NO: 51 - protein, 328 aa, Artificial Sequence
  an artificially synthesized sequence
ASTKGPSVFPLAPSSKSTSGGTAALGCLVKDYFPEPVTVSWNSGALTSGVHTFPAVLQSSGLYSLSSVVTVPSSSLGTQTYICNVNHKPSNTKVDKKVEPKSCDKTHTCPPCPAPELLGGPSVFLFPPKPKDTLMISRTPEVTCVVVDVSHEDPEVKFNWYVDGVEVHNAKTKPREELYNSTYRVVSVLTVLHQDWLNGKEYKCKVSNSALPYPIEKTISKAKGQPREPQVYTLPPSRDELTKNQVSLTCLVKGFYPSDIAVEWESNGQPENNYKTTPPVLDSDGSFFLYSKLTVDKSRWQQGNVFSCSVMHEALHNHYTQKSLSLSP

SEQ ID NO: 52 - protein, 328 aa, Artificial Sequence
  an artificially synthesized sequence
ASTKGPSVFPLAPSSKSTSGGTAALGCLVKDYFPEPVTVSWNSGALTSGVHTFPAVLQSSGLYSLSSVVTVPSSSLGTQTYICNVNHKPSNTKVDKKVEPKSCDKTHTCPPCPAPELLGGPSVFLFPPKPKDTLMISRTPEVTCVVVDVSHEDPEVKFNWYVDGVEVHNAKTKPREELYNSTYRVVSVLTVLHQDWLNGKEYKCKVSNAALPHPIEKTISKAKGQPREPQVYTLPPSRDELTKNQVSLTCLVKGFYPSDIAVEWESNGQPENNYKTTPPVLDSDGSFFLYSKLTVDKSRWQQGNVFSCSVMHEALHNHYTQKSLSLSP

SEQ ID NO: 53 - protein, 328 aa, Artificial Sequence
  an artificially synthesized sequence
ASTKGPSVFPLAPSSKSTSGGTAALGCLVKDYFPEPVTVSWNSGALTSGVHTFPAVLQSSGLYSLSSVVTVPSSSLGTQTYICNVNHKPSNTKVDKKVEPKSCDKTHTCPPCPAPEKKGGPKVFLFPPKPKDTLMISRTPEVTCVVVDVSKEFPEVKFNWYVDGVEVHNAKTKPREEMGNGTYRVVSVLTVLHQDWLNGKEYKCKVSGKALPAPIEKTISKAKGQPREPQVYTLPPSRDELTKNQVSLTCLVKGFYPSDIAVEWESNGQPENNYKTTPPVLDSDGSFFLYSKLTVDKSRWQQGNVFSCSVMHEALHNHYTQKSLSLSP

SEQ ID NO: 54 - protein, 328 aa, Artificial Sequence
  an artificially synthesized sequence
ASTKGPSVFPLAPSSKSTSGGTAALGCLVKDYFPEPVTVSWNSGALTSGVHTFPAVLQSSGLYSLSSVVTVPSSSLGTQTYICNVNHKPSNTKVDKKVEPKSCDKTHTCPPCPAPEKKGGPKVFLFPPKPKDTLMISRTPEVTCVVVDVSKEFPEVKFNWYVDGVEVHNAKTKPREEMGNGTYRVVSVLTVLHQDWLNGKEYKCKVSHKALPAPIEKTISKAKGQPREPQVYTLPPSRDELTKNQVSLTCLVKGFYPSDIAVEWESNGQPENNYKTTPPVLDSDGSFFLYSKLTVDKSRWQQGNVFSCSVMHEALHNHYTQKSLSLSP

SEQ ID NO: 55 - protein, 328 aa, Artificial Sequence
  an artificially synthesized sequence
ASTKGPSVFPLAPSSKSTSGGTAALGCLVKDYFPEPVTVSWNSGALTSGVHTFPAVLQSSGLYSLSSVVTVPSSSLGTQTYICNVNHKPSNTKVDKKVEPKSCDKTHTCPPCPAPEKKGGPKVFLFPPKPKDTLMISRTPEVTCVVVDVSHEDPEVKFNWYVDGVEVHNAKTKPREEMGNGTYRVVSVLTVLHQDWLNGKEYKCKVSGKALPAPIEKTISKAKGQPREPQVYTLPPSRDELTKNQVSLTCLVKGFYPSDIAVEWESNGQPENNYKTTPPVLDSDGSFFLYSKLTVDKSRWQQGNVFSCSVMHEALHNHYTQKSLSLSP

SEQ ID NO: 56 - protein, 328 aa, Artificial Sequence
  an artificially synthesized sequence
ASTKGPSVFPLAPSSKSTSGGTAALGCLVKDYFPEPVTVSWNSGALTSGVHTFPAVLQSSGLYSLSSVVTVPSSSLGTQTYICNVNHKPSNTKVDKKVEPKSCDKTHTCPPCPAPEKKGGPKVFLFPPKPKDTLMISRTPEVTCVVVDVSHEDPEVKFNWYVDGVEVHNAKTKPREEMGNGTYRVVSVLTVLHQDWLNGKEYKCKVSHKALPAPIEKTISKAKGQPREPQVYTLPPSRDELTKNQVSLTCLVKGFYPSDIAVEWESNGQPENNYKTTPPVLDSDGSFFLYSKLTVDKSRWQQGNVFSCSVMHEALHNHYTQKSLSLSP

SEQ ID NO: 57 - protein, 328 aa, Artificial Sequence
  an artificially synthesized sequence
ASTKGPSVFPLAPSSKSTSGGTAALGCLVKDYFPEPVTVSWNSGALTSGVHTFPAVLQSSGLYSLSSVVTVPSSSLGTQTYICNVNHKPSNTKVDKKVEPKSCDKTHTCPPCPAPEKKGGPSVFLFPPKPKDTLMISRTPEVTCVVVDVSKEFPEVKFNWYVDGVEVHNAKTKPREEMGNGTYRVVSVLTVLHQDWLNGKEYKCKVSGKALPAPIEKTISKAKGQPREPQVYTLPPSRDELTKNQVSLTCLVKGFYPSDIAVEWESNGQPENNYKTTPPVLDSDGSFFLYSKLTVDKSRWQQGNVFSCSVMHEALHNHYTQKSLSLSP

SEQ ID NO: 58 - protein, 328 aa, Artificial Sequence
  an artificially synthesized sequence
ASTKGPSVFPLAPSSKSTSGGTAALGCLVKDYFPEPVTVSWNSGALTSGVHTFPAVLQSSGLYSLSSVVTVPSSSLGTQTYICNVNHKPSNTKVDKKVEPKSCDKTHTCPPCPAPEKKGGPSVFLFPPKPKDTLMISRTPEVTCVVVDVSKEFPEVKFNWYVDGVEVHNAKTKPREEMGNGTYRVVSVLTVLHQDWLNGKEYKCKVSHKALPAPIEKTISKAKGQPREPQVYTLPPSRDELTKNQVSLTCLVKGFYPSDIAVEWESNGQPENNYKTTPPVLDSDGSFFLYSKLTVDKSRWQQGNVFSCSVMHEALHNHYTQKSLSLSP

SEQ ID NO: 59 - protein, 328 aa, Artificial Sequence
  an artificially synthesized sequence
ASTKGPSVFPLAPSSKSTSGGTAALGCLVKDYFPEPVTVSWNSGALTSGVHTFPAVLQSSGLYSLSSVVTVPSSSLGTQTYICNVNHKPSNTKVDKKVEPKSCDKTHTCPPCPAPEKKGGPSVFLFPPKPKDTLMISRTPEVTCVVVDVSHEDPEVKFNWYVDGVEVHNAKTKPREEMGNGTYRVVSVLTVLHQDWLNGKEYKCKVSGKALPAPIEKTISKAKGQPREPQVYTLPPSRDELTKNQVSLTCLVKGFYPSDIAVEWESNGQPENNYKTTPPVLDSDGSFFLYSKLTVDKSRWQQGNVFSCSVMHEALHNHYTQKSLSLSP

SEQ ID NO: 60 - protein, 328 aa, Artificial Sequence
  an artificially synthesized sequence
ASTKGPSVFPLAPSSKSTSGGTAALGCLVKDYFPEPVTVSWNSGALTSGVHTFPAVLQSSGLYSLSSVVTVPSSSLGTQTYICNVNHKPSNTKVDKKVEPKSCDKTHTCPPCPAPEKKGGPSVFLFPPKPKDTLMISRTPEVTCVVVDVSHEDPEVKFNWYVDGVEVHNAKTKPREEMGNGTYRVVSVLTVLHQDWLNGKEYKCKVSHKALPAPIEKTISKAKGQPREPQVYTLPPSRDELTKNQVSLTCLVKGFYPSDIAVEWESNGQPENNYKTTPPVLDSDGSFFLYSKLTVDKSRWQQGNVFSCSVMHEALHNHYTQKSLSLSP

SEQ ID NO: 61 - protein, 328 aa, Artificial Sequence
  an artificially synthesized sequence
ASTKGPSVFPLAPSSKSTSGGTAALGCLVKDYFPEPVTVSWNSGALTSGVHTFPAVLQSSGLYSLSSVVTVPSSSLGTQTYICNVNHKPSNTKVDKKVEPKSCDKTHTCPPCPAPEKRGGPKVFLFPPKPKDTLMISRTPEVTCVVVDVSKEFPEVKFNWYVDGVEVHNAKTKPREEMGNGTYRVVSVLTVLHQDWLNGKEYKCKVSGKALPAPIEKTISKAKGQPREPQVYTLPPSRDELTKNQVSLTCLVKGFYPSDIAVEWESNGQPENNYKTTPPVLDSDGSFFLYSKLTVDKSRWQQGNVFSCSVMHEALHNHYTQKSLSLSP

SEQ ID NO: 62 - protein, 328 aa, Artificial Sequence
  an artificially synthesized sequence
ASTKGPSVFPLAPSSKSTSGGTAALGCLVKDYFPEPVTVSWNSGALTSGVHTFPAVLQSSGLYSLSSVVTVPSSSLGTQTYICNVNHKPSNTKVDKKVEPKSCDKTHTCPPCPAPEKRGGPKVFLFPPKPKDTLMISRTPEVTCVVVDVSKEFPEVKFNWYVDGVEVHNAKTKPREEMGNGTYRVVSVLTVLHQDWLNGKEYKCKVSHKALPAPIEKTISKAKGQPREPQVYTLPPSRDELTKNQVSLTCLVKGFYPSDIAVEWESNGQPENNYKTTPPVLDSDGSFFLYSKLTVDKSRWQQGNVFSCSVMHEALHNHYTQKSLSLSP

SEQ ID NO: 63 - protein, 328 aa, Artificial Sequence
  an artificially synthesized sequence
ASTKGPSVFPLAPSSKSTSGGTAALGCLVKDYFPEPVTVSWNSGALTSGVHTFPAVLQSSGLYSLSSVVTVPSSSLGTQTYICNVNHKPSNTKVDKKVEPKSCDKTHTCPPCPAPEKRGGPKVFLFPPKPKDTLMISRTPEVTCVVVDVSHEDPEVKFNWYVDGVEVHNAKTKPREEMGNGTYRVVSVLTVLHQDWLNGKEYKCKVSGKALPAPIEKTISKAKGQPREPQVYTLPPSRDELTKNQVSLTCLVKGFYPSDIAVEWESNGQPENNYKTTPPVLDSDGSFFLYSKLTVDKSRWQQGNVFSCSVMHEALHNHYTQKSLSLSP

SEQ ID NO: 64 - protein, 328 aa, Artificial Sequence
  an artificially synthesized sequence
ASTKGPSVFPLAPSSKSTSGGTAALGCLVKDYFPEPVTVSWNSGALTSGVHTFPAVLQSSGLYSLSSVVTVPSSSLGTQTYICNVNHKPSNTKVDKKVEPKSCDKTHTCPPCPAPEKRGGPKVFLFPPKPKDTLMISRTPEVTCVVVDVSHEDPEVKFNWYVDGVEVHNAKTKPREEMGNGTYRVVSVLTVLHQDWLNGKEYKCKVSHKALPAPIEKTISKAKGQPREPQVYTLPPSRDELTKNQVSLTCLVKGFYPSDIAVEWESNGQPENNYKTTPPVLDSDGSFFLYSKLTVDKSRWQQGNVFSCSVMHEALHNHYTQKSLSLSP

SEQ ID NO: 65 - protein, 328 aa, Artificial Sequence
  an artificially synthesized sequence
ASTKGPSVFPLAPSSKSTSGGTAALGCLVKDYFPEPVTVSWNSGALTSGVHTFPAVLQSSGLYSLSSVVTVPSSSLGTQTYICNVNHKPSNTKVDKKVEPKSCDKTHTCPPCPAPEKRGGPSVFLFPPKPKDTLMISRTPEVTCVVVDVSKEFPEVKFNWYVDGVEVHNAKTKPREEMGNGTYRVVSVLTVLHQDWLNGKEYKCKVSGKALPAPIEKTISKAKGQPREPQVYTLPPSRDELTKNQVSLTCLVKGFYPSDIAVEWESNGQPENNYKTTPPVLDSDGSFFLYSKLTVDKSRWQQGNVFSCSVMHEALHNHYTQKSLSLSP

SEQ ID NO: 66 - protein, 328 aa, Artificial Sequence
  an artificially synthesized sequence
ASTKGPSVFPLAPSSKSTSGGTAALGCLVKDYFPEPVTVSWNSGALTSGVHTFPAVLQSSGLYSLSSVVTVPSSSLGTQTYICNVNHKPSNTKVDKKVEPKSCDKTHTCPPCPAPEKRGGPSVFLFPPKPKDTLMISRTPEVTCVVVDVSKEFPEVKFNWYVDGVEVHNAKTKPREEMGNGTYRVVSVLTVLHQDWLNGKEYKCKVSHKALPAPIEKTISKAKGQPREPQVYTLPPSRDELTKNQVSLTCLVKGFYPSDIAVEWESNGQPENNYKTTPPVLDSDGSFFLYSKLTVDKSRWQQGNVFSCSVMHEALHNHYTQKSLSLSP

SEQ ID NO: 67 - protein, 328 aa, Artificial Sequence
  an artificially synthesized sequence
ASTKGPSVFPLAPSSKSTSGGTAALGCLVKDYFPEPVTVSWNSGALTSGVHTFPAVLQSSGLYSLSSVVTVPSSSLGTQTYICNVNHKPSNTKVDKKVEPKSCDKTHTCPPCPAPEKRGGPSVFLFPPKPKDTLMISRTPEVTCVVVDVSHEDPEVKFNWYVDGVEVHNAKTKPREEMGNGTYRVVSVLTVLHQDWLNGKEYKCKVSGKALPAPIEKTISKAKGQPREPQVYTLPPSRDELTKNQVSLTCLVKGFYPSDIAVEWESNGQPENNYKTTPPVLDSDGSFFLYSKLTVDKSRWQQGNVFSCSVMHEALHNHYTQKSLSLSP

SEQ ID NO: 68 - protein, 328 aa, Artificial Sequence
  an artificially synthesized sequence
ASTKGPSVFPLAPSSKSTSGGTAALGCLVKDYFPEPVTVSWNSGALTSGVHTFPAVLQSSGLYSLSSVVTVPSSSLGTQTYICNVNHKPSNTKVDKKVEPKSCDKTHTCPPCPAPEKRGGPSVFLFPPKPKDTLMISRTPEVTCVVVDVSHEDPEVKFNWYVDGVEVHNAKTKPREEMGNGTYRVVSVLTVLHQDWLNGKEYKCKVSHKALPAPIEKTISKAKGQPREPQVYTLPPSRDELTKNQVSLTCLVKGFYPSDIAVEWESNGQPENNYKTTPPVLDSDGSFFLYSKLTVDKSRWQQGNVFSCSVMHEALHNHYTQKSLSLSP

SEQ ID NO: 69 - protein, 328 aa, Artificial Sequence
  an artificially synthesized sequence
ASTKGPSVFPLAPSSKSTSGGTAALGCLVKDYFPEPVTVSWNSGALTSGVHTFPAVLQSSGLYSLSSVVTVPSSSLGTQTYICNVNHKPSNTKVDKKVEPKSCDKTHTCPPCPAPELLGGPSVFLFPPKVKDTLMISRTPEVTCVVVDVSHEDPEVKFNWYVDGVEVHNAKTKPREEQYNSTYRVVSVLTVLHQDWLNGKEYKCKVSNKALPAPIEKTISKAKGQPREPQVYTLPPSRDELTKNQVSLTCLVKGFYPSDIAVEWESNGQPENNYKTTPPVLDSDGSFFLYSKLTVDKSRWQQGNVFSCSVMHEALHNHYTQKSLSLSP

SEQ ID NO: 70 - protein, 328 aa, Artificial Sequence
  an artificially synthesized sequence
ASTKGPSVFPLAPSSKSTSGGTAALGCLVKDYFPEPVTVSWNSGALTSGVHTFPAVLQSSGLYSLSSVVTVPSSSLGTQTYICNVNHKPSNTKVDKKVEPKSCDKTHTCPPCPAPELLGGPSVFLFPPKPKDFLMISRTPEVTCVVVDVSHEDPEVKFNWYVDGVEVHNAKTKPREEQYNSTYRVVSVLTVLHQDWLNGKEYKCKVSNKALPAPIEKTISKAKGQPREPQVYTLPPSRDELTKNQVSLTCLVKGFYPSDIAVEWESNGQPENNYKTTPPVLDSDGSFFLYSKLTVDKSRWQQGNVFSCSVMHEALHNHYTQKSLSLSP

SEQ ID NO: 71 - protein, 328 aa, Artificial Sequence
  an artificially synthesized sequence
ASTKGPSVFPLAPSSKSTSGGTAALGCLVKDYFPEPVTVSWNSGALTSGVHTFPAVLQSSGLYSLSSVVTVPSSSLGTQTYICNVNHKPSNTKVDKKVEPKSCDKTHTCPPCPAPELLGGPSVFLFPPKPKDILMISRTPEVTCVVVDVSHEDPEVKFNWYVDGVEVHNAKTKPREEQYNSTYRVVSVLTVLHQDWLNGKEYKCKVSNKALPAPIEKTISKAKGQPREPQVYTLPPSRDELTKNQVSLTCLVKGFYPSDIAVEWESNGQPENNYKTTPPVLDSDGSFFLYSKLTVDKSRWQQGNVFSCSVMHEALHNHYTQKSLSLSP

SEQ ID NO: 72 - protein, 328 aa, Artificial Sequence
  an artificially synthesized sequence
ASTKGPSVFPLAPSSKSTSGGTAALGCLVKDYFPEPVTVSWNSGALTSGVHTFPAVLQSSGLYSLSSVVTVPSSSLGTQTYICNVNHKPSNTKVDKKVEPKSCDKTHTCPPCPAPELLGGPSVFLFPPKPKDMLMISRTPEVTCVVVDVSHEDPEVKFNWYVDGVEVHNAKTKPREEQYNSTYRVVSVLTVLHQDWLNGKEYKCKVSNKALPAPIEKTISKAKGQPREPQVYTLPPSRDELTKNQVSLTCLVKGFYPSDIAVEWESNGQPENNYKTTPPVLDSDGSFFLYSKLTVDKSRWQQGNVFSCSVMHEALHNHYTQKSLSLSP

SEQ ID NO: 73 - protein, 328 aa, Artificial Sequence
  an artificially synthesized sequence
ASTKGPSVFPLAPSSKSTSGGTAALGCLVKDYFPEPVTVSWNSGALTSGVHTFPAVLQSSGLYSLSSVVTVPSSSLGTQTYICNVNHKPSNTKVDKKVEPKSCDKTHTCPPCPAPELLGGPSVFLFPPKPKDVLMISRTPEVTCVVVDVSHEDPEVKFNWYVDGVEVHNAKTKPREEQYNSTYRVVSVLTVLHQDWLNGKEYKCKVSNKALPAPIEKTISKAKGQPREPQVYTLPPSRDELTKNQVSLTCLVKGFYPSDIAVEWESNGQPENNYKTTPPVLDSDGSFFLYSKLTVDKSRWQQGNVFSCSVMHEALHNHYTQKSLSLSP

SEQ ID NO: 74 - protein, 328 aa, Artificial Sequence
  an artificially synthesized sequence
ASTKGPSVFPLAPSSKSTSGGTAALGCLVKDYFPEPVTVSWNSGALTSGVHTFPAVLQSSGLYSLSSVVTVPSSSLGTQTYICNVNHKPSNTKVDKKVEPKSCDKTHTCPPCPAPELLGGPSVFLFPPKPKDWLMISRTPEVTCVVVDVSHEDPEVKFNWYVDGVEVHNAKTKPREEQYNSTYRVVSVLTVLHQDWLNGKEYKCKVSNKALPAPIEKTISKAKGQPREPQVYTLPPSRDELTKNQVSLTCLVKGFYPSDIAVEWESNGQPENNYKTTPPVLDSDGSFFLYSKLTVDKSRWQQGNVFSCSVMHEALHNHYTQKSLSLSP

SEQ ID NO: 75 - protein, 328 aa, Artificial Sequence
  an artificially synthesized sequence
ASTKGPSVFPLAPSSKSTSGGTAALGCLVKDYFPEPVTVSWNSGALTSGVHTFPAVLQSSGLYSLSSVVTVPSSSLGTQTYICNVNHKPSNTKVDKKVEPKSCDKTHTCPPCPAPELLGGPSVFLFPPKPKDYLMISRTPEVTCVVVDVSHEDPEVKFNWYVDGVEVHNAKTKPREEQYNSTYRVVSVLTVLHQDWLNGKEYKCKVSNKALPAPIEKTISKAKGQPREPQVYTLPPSRDELTKNQVSLTCLVKGFYPSDIAVEWESNGQPENNYKTTPPVLDSDGSFFLYSKLTVDKSRWQQGNVFSCSVMHEALHNHYTQKSLSLSP

SEQ ID NO: 76 - protein, 328 aa, Artificial Sequence
  an artificially synthesized sequence
ASTKGPSVFPLAPSSKSTSGGTAALGCLVKDYFPEPVTVSWNSGALTSGVHTFPAVLQSSGLYSLSSVVTVPSSSLGTQTYICNVNHKPSNTKVDKKVEPKSCDKTHTCPPCPAPELLGGPSVFLFPPKPKDTLMISRTPEVTCVVVDVSHEDPEVKFNWYVDGVEVHNAKTKPREEQYNGTYRVVSVLTVLHQDWLNGKEYKCKVSNKALPAPIEKTISKAKGQPREPQVYTLPPSRDELTKNQVSLTCLVKGFYPSDIAVEWESNGQPENNYKTTPPVLDSDGSFFLYSKLTVDKSRWQQGNVFSCSVMHEALHNHYTQKSLSLSP

SEQ ID NO: 77 - protein, 328 aa, Artificial Sequence
  an artificially synthesized sequence
ASTKGPSVFPLAPSSKSTSGGTAALGCLVKDYFPEPVTVSWNSGALTSGVHTFPAVLQSSGLYSLSSVVTVPSSSLGTQTYICNVNHKPSNTKVDKKVEPKSCDKTHTCPPCPAPELLGGPSVFLFPPKPKDTLMISRTPEVTCVVVDVSHEDPEVKFNWYVDGVEVHNAKTKPREEQYNSTYRVVSVLAVLHQDWLNGKEYKCKVSNKALPAPIEKTISKAKGQPREPQVYTLPPSRDELTKNQVSLTCLVKGFYPSDIAVEWESNGQPENNYKTTPPVLDSDGSFFLYSKLTVDKSRWQQGNVFSCSVMHEALHNHYTQKSLSLSP

SEQ ID NO: 78 - protein, 328 aa, Artificial Sequence
  an artificially synthesized sequence
ASTKGPSVFPLAPSSKSTSGGTAALGCLVKDYFPEPVTVSWNSGALTSGVHTFPAVLQSSGLYSLSSVVTVPSSSLGTQTYICNVNHKPSNTKVDKKVEPKSCDKTHTCPPCPAPELLGGPSVFLFPPKPKDTLMISRTPEVTCVVVDVSHEDPEVKFNWYVDGVEVHNAKTKPREEQYNSTYRVVSVLQVLHQDWLNGKEYKCKVSNKALPAPIEKTISKAKGQPREPQVYTLPPSRDELTKNQVSLTCLVKGFYPSDIAVEWESNGQPENNYKTTPPVLDSDGSFFLYSKLTVDKSRWQQGNVFSCSVMHEALHNHYTQKSLSLSP

SEQ ID NO: 79 - protein, 328 aa, Artificial Sequence
  an artificially synthesized sequence
ASTKGPSVFPLAPSSKSTSGGTAALGCLVKDYFPEPVTVSWNSGALTSGVHTFPAVLQSSGLYSLSSVVTVPSSSLGTQTYICNVNHKPSNTKVDKKVEPKSCDKTHTCPPCPAPELLGGPSVFLFPPKPKDTLMISRTPEVTCVVVDVSHEDPEVKFNWYVDGVEVHNAKTKPREEQYNSTYRVVSVLPVLHQDWLNGKEYKCKVSNKALPAPIEKTISKAKGQPREPQVYTLPPSRDELTKNQVSLTCLVKGFYPSDIAVEWESNGQPENNYKTTPPVLDSDGSFFLYSKLTVDKSRWQQGNVFSCSVMHEALHNHYTQKSLSLSP

SEQ ID NO: 80 - protein, 328 aa, Artificial Sequence
  an artificially synthesized sequence
ASTKGPSVFPLAPSSKSTSGGTAALGCLVKDYFPEPVTVSWNSGALTSGVHTFPAVLQSSGLYSLSSVVTVPSSSLGTQTYICNVNHKPSNTKVDKKVEPKSCDKTHTCPPCPAPELLGGPSVFLFPPKPKDTLMISRTPEVTCVVVDVSHEDPEVKFNWYVDGVEVHNAKTKPREEQYNSTYRVVSVLTVAHQDWLNGKEYKCKVSNKALPAPIEKTISKAKGQPREPQVYTLPPSRDELTKNQVSLTCLVKGFYPSDIAVEWESNGQPENNYKTTPPVLDSDGSFFLYSKLTVDKSRWQQGNVFSCSVMHEALHNHYTQKSLSLSP

SEQ ID NO: 81 - protein, 328 aa, Artificial Sequence
  an artificially synthesized sequence
ASTKGPSVFPLAPSSKSTSGGTAALGCLVKDYFPEPVTVSWNSGALTSGVHTFPAVLQSSGLYSLSSVVTVPSSSLGTQTYICNVNHKPSNTKVDKKVEPKSCDKTHTCPPCPAPELLGGPSVFLFPPKPKDTLMISRTPEVTCVVVDVSHEDPEVKFNWYVDGVEVHNAKTKPREEQYNSTYRVVSVLTVDHQDWLNGKEYKCKVSNKALPAPIEKTISKAKGQPREPQVYTLPPSRDELTKNQVSLTCLVKGFYPSDIAVEWESNGQPENNYKTTPPVLDSDGSFFLYSKLTVDKSRWQQGNVFSCSVMHEALHNHYTQKSLSLSP

SEQ ID NO: 82 - protein, 328 aa, Artificial Sequence
  an artificially synthesized sequence
ASTKGPSVFPLAPSSKSTSGGTAALGCLVKDYFPEPVTVSWNSGALTSGVHTFPAVLQSSGLYSLSSVVTVPSSSLGTQTYICNVNHKPSNTKVDKKVEPKSCDKTHTCPPCPAPELLGGPSVFLFPPKPKDTLMISRTPEVTCVVVDVSHEDPEVKFNWYVDGVEVHNAKTKPREEQYNSTYRVVSVLTVRHQDWLNGKEYKCKVSNKALPAPIEKTISKAKGQPREPQVYTLPPSRDELTKNQVSLTCLVKGFYPSDIAVEWESNGQPENNYKTTPPVLDSDGSFFLYSKLTVDKSRWQQGNVFSCSVMHEALHNHYTQKSLSLSP

SEQ ID NO: 83 - protein, 328 aa, Artificial Sequence
  an artificially synthesized sequence
ASTKGPSVFPLAPSSKSTSGGTAALGCLVKDYFPEPVTVSWNSGALTSGVHTFPAVLQSSGLYSLSSVVTVPSSSLGTQTYICNVNHKPSNTKVDKKVEPKSCDKTHTCPPCPAPELLGGPSVFLFPPKPKDTLMISRTPEVTCVVVDVSHEDPEVKFNWYVDGVEVHNAKTKPREEQYNSTYRVVSVLTVPHQDWLNGKEYKCKVSNKALPAPIEKTISKAKGQPREPQVYTLPPSRDELTKNQVSLTCLVKGFYPSDIAVEWESNGQPENNYKTTPPVLDSDGSFFLYSKLTVDKSRWQQGNVFSCSVMHEALHNHYTQKSLSLSP

SEQ ID NO: 84 - protein, 328 aa, Artificial Sequence
  an artificially synthesized sequence
ASTKGPSVFPLAPSSKSTSGGTAALGCLVKDYFPEPVTVSWNSGALTSGVHTFPAVLQSSGLYSLSSVVTVPSSSLGTQTYICNVNHKPSNTKVDKKVEPKSCDKTHTCPPCPAPELLGGPSVFLFPPKPKDTLMISRTPEVTCVVVDVSHEDPEVKFNWYVDGVEVHNAKTKPREEQYNSTYRVVSVLTVLHQDWLAGKEYKCKVSNKALPAPIEKTISKAKGQPREPQVYTLPPSRDELTKNQVSLTCLVKGFYPSDIAVEWESNGQPENNYKTTPPVLDSDGSFFLYSKLTVDKSRWQQGNVFSCSVMHEALHNHYTQKSLSLSP

SEQ ID NO: 85 - protein, 328 aa, Artificial Sequence
  an artificially synthesized sequence
ASTKGPSVFPLAPSSKSTSGGTAALGCLVKDYFPEPVTVSWNSGALTSGVHTFPAVLQSSGLYSLSSVVTVPSSSLGTQTYICNVNHKPSNTKVDKKVEPKSCDKTHTCPPCPAPELLGGPSVFLFPPKPKDTLMISRTPEVTCVVVDVSHEDPEVKFNWYVDGVEVHNAKTKPREEQYNSTYRVVSVLTVLHQDWLNGKEYKCKVSNKALPAPIEKTISKAKGQPREPQVYTLPPSRDELTHNQVSLTCLVKGFYPSDIAVEWESNGQPENNYKTTPPVLDSDGSFFLYSKLTVDKSRWQQGNVFSCSVMHEALHNHYTQKSLSLSP

SEQ ID NO: 86 - protein, 328 aa, Artificial Sequence
  an artificially synthesized sequence
ASTKGPSVFPLAPSSKSTSGGTAALGCLVKDYFPEPVTVSWNSGALTSGVHTFPAVLQSSGLYSLSSVVTVPSSSLGTQTYICNVNHKPSNTKVDKKVEPKSCDKTHTCPPCPAPELLGGPSVFLFPPKPKDTLMISRTPEVTCVVVDVSHEDPEVKFNWYVDGVEVHNAKTKPREEQYNSTYRVVSVLTVLHQDWLNGKEYKCKVSNKALPAPIEKTISKAKGQPREPQVYTLPPSRDELTKNQVSLTCLVKGFYPSDIAVEWESNDPPESNYKTTPPVLDSDGSFFLYSKLTVDKSRWQQGNVFSCSVMHEALHNHYTQKSLSLSP

SEQ ID NO: 87 - protein, 328 aa, Artificial Sequence
  an artificially synthesized sequence
ASTKGPSVFPLAPSSKSTSGGTAALGCLVKDYFPEPVTVSWNSGALTSGVHTFPAVLQSSGLYSLSSVVTVPSSSLGTQTYICNVNHKPSNTKVDKKVEPKSCDKTHTCPPCPAPELLGGPSVFLFPPKPKDTLMISRTPEVTCVVVDVSHEDPEVKFNWYVDGVEVHNAKTKPREEQYNSTYRVVSVLTVLHQDWLNGKEYKCKVSNKALPAPIEKTISKAKGQPREPQVYTLPPSRDELTKNQVSLTCLVKGFYPSDIAVEWESNGQEENNYKTTPPVLDSDGSFFLYSKLTVDKSRWQQGNVFSCSVMHEALHNHYTQKSLSLSP

SEQ ID NO: 88 - protein, 328 aa, Artificial Sequence
  an artificially synthesized sequence
ASTKGPSVFPLAPSSKSTSGGTAALGCLVKDYFPEPVTVSWNSGALTSGVHTFPAVLQSSGLYSLSSVVTVPSSSLGTQTYICNVNHKPSNTKVDKKVEPKSCDKTHTCPPCPAPELLGGPSVFLFPPKPKDTLMISRTPEVTCVVVDVSHEDPEVKFNWYVDGVEVHNAKTKPREEQYNSTYRVVSVLTVLHQDWLNGKEYKCKVSNKALPAPIEKTISKAKGQPREPQVYTLPPSRDELTKNQVSLTCLVKGFYPSDIAVEWESNGQPENNYKTTPPVLDSDGSFFLYSKLTVDKSRWQQGNVFSCSVHHEALHNHYTQKSLSLSP

SEQ ID NO: 89 - protein, 328 aa, Artificial Sequence
  an artificially synthesized sequence
ASTKGPSVFPLAPSSKSTSGGTAALGCLVKDYFPEPVTVSWNSGALTSGVHTFPAVLQSSGLYSLSSVVTVPSSSLGTQTYICNVNHKPSNTKVDKKVEPKSCDKTHTCPPCPAPELLGGPSVFLFPPKPKDTLMISRTPEVTCVVVDVSHEDPEVKFNWYVDGVEVHNAKTKPREEQYNSTYRVVSVLTVLHQDWLNGKEYKCKVSNKALPAPIEKTISKAKGQPREPQVYTLPPSRDELTKNQVSLTCLVKGFYPSDIAVEWESNGQPENNYKTTPPVLDSDGSFFLYSKLTVDKSRWQQGNVFSCSVWHEALHNHYTQKSLSLSP

SEQ ID NO: 90 - protein, 328 aa, Artificial Sequence
  an artificially synthesized sequence
ASTKGPSVFPLAPSSKSTSGGTAALGCLVKDYFPEPVTVSWNSGALTSGVHTFPAVLQSSGLYSLSSVVTVPSSSLGTQTYICNVNHKPSNTKVDKKVEPKSCDKTHTCPPCPAPELLGGPSVFLFPPKPKDTLMISRTPEVTCVVVDVSHEDPEVKFNWYVDGVEVHNAKTKPREEQYNSTYRVVSVLTVLHQDWLNGKEYKCKVSNKALPAPIEKTISKAKGQPREPQVYTLPPSRDELTKNQVSLTCLVKGFYPSDIAVEWESNGQPENNYKTTPPVLDSDGSFFLYSKLTVDKSRWQQGNVFSCSVYHEALHNHYTQKSLSLSP

SEQ ID NO: 91 - protein, 328 aa, Artificial Sequence
  an artificially synthesized sequence
ASTKGPSVFPLAPSSKSTSGGTAALGCLVKDYFPEPVTVSWNSGALTSGVHTFPAVLQSSGLYSLSSVVTVPSSSLGTQTYICNVNHKPSNTKVDKKVEPKSCDKTHTCPPCPAPELLGGPSVFLFPPKPKDTLMISRTPEVTCVVVDVSHEDPEVKFNWYVDGVEVHNAKTKPREEQYNSTYRVVSVLTVLHQDWLNGKEYKCKVSNKALPAPIEKTISKAKGQPREPQVYTLPPSRDELTKNQVSLTCLVKGFYPSDIAVEWESNGQPENNYKTTPPVLDSDGSFFLYSKLTVDKSRWQQGNVFSCSVFHEALHNHYTQKSLSLSP

SEQ ID NO: 92 - protein, 328 aa, Artificial Sequence
  an artificially synthesized sequence
ASTKGPSVFPLAPSSKSTSGGTAALGCLVKDYFPEPVTVSWNSGALTSGVHTFPAVLQSSGLYSLSSVVTVPSSSLGTQTYICNVNHKPSNTKVDKKVEPKSCDKTHTCPPCPAPELLGGPSVFLFPPKPKDTLMISRTPEVTCVVVDVSHEDPEVKFNWYVDGVEVHNAKTKPREEQYNSTYRVVSVLTVLHQDWLNGKEYKCKVSNKALPAPIEKTISKAKGQPREPQVYTLPPSRDELTKNQVSLTCLVKGFYPSDIAVEWESNGQPENNYKTTPPVLDSDGSFFLYSKLTVDKSRWQQGNVFSCSVMHEALKNHYTQKSLSLSP